European Patent Application EP 4 155 390 A1, published March 29, 2023. Title: SERUM-FREE INDUCTION METHOD FOR SENSORY NEURON CELL. Applicant: IREGENE THERAPEUTICS LTD. Application EP20936500.6. The sequence listing filed with the application follows.

SEQUENCE LISTING (44 sequences)

SEQ ID NO: 1 - DNA, 23 bp, Artificial sequence
  misc_feature (1)..(23): forward primer for amplification of SOX10
ccacctatgccacagtgcctaag

SEQ ID NO: 2 - DNA, 22 bp, Artificial sequence
  misc_feature (1)..(22): reverse primer for amplification of SOX10
gtgccaactccttcctgccttc

SEQ ID NO: 3 - DNA, 24 bp, Artificial sequence
  misc_feature (1)..(24): forward primer for amplification of SCN9A
aagaggatgtgtctgctactgtca

SEQ ID NO: 4 - DNA, 22 bp, Artificial sequence
  misc_feature (1)..(22): reverse primer for amplification of SCN9A
gaaggtggagaggtggtggatg

SEQ ID NO: 5 - DNA, 23 bp, Artificial sequence
  misc_feature (1)..(23): forward primer for amplification of SCN10A
aacttccagaccttcgccaacag

SEQ ID NO: 6 - DNA, 24 bp, Artificial sequence
  misc_feature (1)..(24): reverse primer for amplification of SCN10A
tggtgaagaagatgatgcctacgg

SEQ ID NO: 7 - DNA, 24 bp, Artificial sequence
  misc_feature (1)..(24): forward primer for amplification of SCN11A
tgatgatgtcgcttccttctctgt

SEQ ID NO: 8 - DNA, 24 bp, Artificial sequence
  misc_feature (1)..(24): reverse primer for amplification of SCN11A
ccaacctgctgatgtgcttatctg

SEQ ID NO: 9 - DNA, 22 bp, Artificial sequence
  misc_feature (1)..(22): forward primer for amplification of Nestin
tcaagatgtccctcagcctgga

SEQ ID NO: 10 - DNA, 23 bp, Artificial sequence
  misc_feature (1)..(23): reverse primer for amplification of Nestin
tggcacaggtgtctcaagggtag

SEQ ID NO: 11 - DNA, 23 bp, Artificial sequence
  misc_feature (1)..(23): forward primer for amplification of CaV2.1
tggaggacgaggacagtgatgaa

SEQ ID NO: 12 - DNA, 23 bp, Artificial sequence
  misc_feature (1)..(23): reverse primer for amplification of CaV2.1
cgagtcaggatgccagagttctt

SEQ ID NO: 13 - DNA, 22 bp, Artificial sequence
  misc_feature (1)..(22): forward primer for amplification of Cav2.2
cagcatcaaccgccacaacaac

SEQ ID NO: 14 - DNA, 24 bp, Artificial sequence
  misc_feature (1)..(24): reverse primer for amplification of Cav2.2
ggagcacaggaagatgaaggagac

SEQ ID NO: 15 - DNA, 22 bp, Artificial sequence
  misc_feature (1)..(22): forward primer for amplification of CaV3.2
gctggtggtggagacgctgata

SEQ ID NO: 16 - DNA, 23 bp, Artificial sequence
  misc_feature (1)..(23): reverse primer for amplification of CaV3.2
actgtgccttggtggagatgttc

SEQ ID NO: 17 - DNA, 22 bp, Artificial sequence
  misc_feature (1)..(22): forward primer for amplification of KV4.3
cctgctgctcccgtcgtagtaa

SEQ ID NO: 18 - DNA, 24 bp, Artificial sequence
  misc_feature (1)..(24): reverse primer for amplification of KV4.3
gatgctgatgatggctgtggtgat

SEQ ID NO: 19 - DNA, 24 bp, Artificial sequence
  misc_feature (1)..(24): forward primer for amplification of KCNIP2
gctccaagttccacaggtctgcta

SEQ ID NO: 20 - DNA, 23 bp, Artificial sequence
  misc_feature (1)..(23): reverse primer for amplification of KCNIP2
caccacaaccaccaccaacacat

SEQ ID NO: 21 - DNA, 24 bp, Artificial sequence
  misc_feature (1)..(24): forward primer for amplification of KV7.2
tgtatgtgtccttgtgccgtagtg

SEQ ID NO: 22 - DNA, 24 bp, Artificial sequence
  misc_feature (1)..(24): reverse primer for amplification of KV7.2
gcatcaacctgtccgtgtgagtaa

SEQ ID NO: 23 - DNA, 24 bp, Artificial sequence
  misc_feature (1)..(24): forward primer for amplification of KV7.3
gcatattcaaccaaagcccgtgta

SEQ ID NO: 24 - DNA, 24 bp, Artificial sequence
  misc_feature (1)..(24): reverse primer for amplification of KV7.3
aaggacctgctgaacagacaagag

SEQ ID NO: 25 - DNA, 23 bp, Artificial sequence
  misc_feature (1)..(23)
  misc_feature (1)..(23): forward primer for amplification of GABRA3
ggactggttcatagccgtctgtt

SEQ ID NO: 26 - DNA, 24 bp, Artificial sequence
  misc_feature (1)..(24): reverse primer for amplification of GABRA3
acgatgttgaaggtagtgctggtt

SEQ ID NO: 27 - DNA, 20 bp, Artificial sequence
  misc_feature (1)..(20): forward primer for amplification of TRPV4
tgccgtgacagcgagacctt

SEQ ID NO: 28 - DNA, 23 bp, Artificial sequence
  misc_feature (1)..(23): reverse primer for amplification of TRPV4
cagatgtgcttgctctccttgga

SEQ ID NO: 29 - DNA, 22 bp, Artificial sequence
  misc_feature (1)..(22): forward primer for amplification of TRPM8
ggcaccgtccaggagaacaatg

SEQ ID NO: 30 - DNA, 24 bp, Artificial sequence
  misc_feature (1)..(24): reverse primer for amplification of TRPM8
gcagcaacacttgaagcacttctt

SEQ ID NO: 31 - DNA, 21 bp, Artificial sequence
  misc_feature (1)..(21): forward primer for amplification of KCa2.1
tggctggaaggcactggtgat

SEQ ID NO: 32 - DNA, 24 bp, Artificial sequence
  misc_feature (1)..(24): reverse primer for amplification of KCa2.1
gctggtacaggtgtccctagagag

SEQ ID NO: 33 - DNA, 24 bp, Artificial sequence
  misc_feature (1)..(24): forward primer for amplification of KCa2.2
ggagtgaagacttcgagaagagga

SEQ ID NO: 34 - DNA, 21 bp, Artificial sequence
  misc_feature (1)..(21): reverse primer for amplification of KCa2.2
tggtggtgctgtggaagagga

SEQ ID NO: 35 - DNA, 24 bp, Artificial sequence
  misc_feature (1)..(24): forward primer for amplification of NR2A
gttggtgatggtgagatggaggag

SEQ ID NO: 36 - DNA, 24 bp, Artificial sequence
  misc_feature (1)..(24): reverse primer for amplification of NR2A
ccagatgaaggtgatgaggctgag

SEQ ID NO: 37 - DNA, 21 bp, Artificial sequence
  misc_feature (1)..(21): forward primer for amplification of NR2B
actactgctgctgctggttca

SEQ ID NO: 38 - DNA, 24 bp, Artificial sequence
  misc_feature (1)..(24): reverse primer for amplification of NR2B
aaggtatgactgagttggctgtga

SEQ ID NO: 39 - DNA, 24 bp, Artificial sequence
  misc_feature (1)..(24): forward primer for amplification of TRPV1
gcagtgccttcttcatccttcctt

SEQ ID NO: 40 - DNA, 22 bp, Artificial sequence
  misc_feature (1)..(22): reverse primer for amplification of TRPV1
aagcatgtgccattgcggagaa

SEQ ID NO: 41 - DNA, 23 bp, Artificial sequence
  misc_feature (1)..(23): forward primer for amplification of CASP3
ggaagcgaatcaatggactctgg

SEQ ID NO: 42 - DNA, 22 bp, Artificial sequence
  misc_feature (1)..(22): reverse primer for amplification of CASP3
gcatcgacatctgtaccagacc

SEQ ID NO: 43 - DNA, 20 bp, Artificial sequence
  misc_feature (1)..(20): forward primer for amplification of ACTIN
tccctggagaagagctacga

SEQ ID NO: 44 - DNA, 20 bp, Artificial sequence
  misc_feature (1)..(20): reverse primer for amplification of ACTIN
agcactgtgttggcgtacag